European Patent Specification EP 3 489 361 B1, published March 8, 2023. Title: Microorganisms having an acyltransferase activity and the use thereof. Applicant: CJ CHEILJEDANG CORPORATION. The sequence listing filed with the application follows.

SEQUENCE LISTING (52 sequences)

SEQ ID NO: 1 - protein, 171 aa, Pseudomonas putida
MSHEIRDALPADVPGILDIYNDAVRNTTAIWNETPVDLGNRQAWFEARAQQGYPILVAVDHSGVLGYASFGDWRPFEGFRNTVEHSVYIRGDQRGKGLGPQLMTALIARARGCGKHVMVAAIESGNAASVRLHERLGFVVTGQMPQVGVKFGRWLDLTFMQLVLDPGAEPA

SEQ ID NO: 2 - protein, 163 aa, Bacillus subtilis
MTLRLAEHRDLEAVVAIYNSTIASRMVTADTEPVTPEDRMEWFSGHTESRPLYVAEDENGNVAAWISFETFYGRPAYNKTAEVSIYIDEACRGKGVGSYLLQEALRIAPNLGIRSLMAFIFGHNKPSLKLFEKHGFAEWGLFPGIAEMDGKRYDLKILGRELS

SEQ ID NO: 3 - protein, 171 aa, Enterobacter sp. 638
MIIRHASKEDCAAIGEIYNHAVVHTAAIWNDTTVDTENRIAWFEARTLMGYPVLVSEENGVVTGYASFGDWRAFDGFRHTVEHSVYVHPDHQGKGIGRELMKALIGEARNIGKHVMVAGIEAQNHGSIHLHKTLGFVITGQMPQVGTKFGRWLDLTFMQLQLDERIDPDAI

SEQ ID NO: 4 - protein, 175 aa, Pseudovibrio sp. FO-BEG1
MKLRQATKSDLPTLLEIHNDAVKTLAAIWTDTLETLEDRVSWFEKRIAGGFPIIVAEDENGDVLGYGSYGSFREKSGYDKTVEHSVYVTPQSRGNGAGSVLLEKLIELAKQDDRHVLIGAIDSENKGSIRLHERYGFRITGELPQVGFKFGRWLDLTLMTLILNDDEAPTALAHE

SEQ ID NO: 5 - protein, 154 aa, Yarrowia lipolytica PO1f
MKISPEPYTADLYKLVRKNMKGMYEGSGMGWNRVDKIDEMEDEELAYHVARENGEMLGFVSFMHTVEDDVEVVYLYELQVAKGRQGHGVGKELMRVVIDEARACGRPIMLTVFLMNERAIGFYRRYGFERVGRGPQEGKRVRGWMQMRRDTRSD

SEQ ID NO: 6 - protein, 179 aa, Corynebacterium glutamicum ATCC 13032
MVERDFTIRPIREGDFPQVRDIYELGLETGHATYETSGPTWDQFSQSKIMDTVMVAVENNDPDFILGWVSAAPISSRQVFHGVVEDSIYIHPQGQGRGIGGALLDALITYCESNGIWSIHSWIFPENLGSAKLHESKGFVKVGTMHQMARMPYGEMEGQWRDCDLWECLLSVPEQAQSS

SEQ ID NO: 7 - DNA, 516 bp, Pseudomonas putida
atgagccatgaaattcgcgatgcgctgccggcggatgtgccgggcattctggatatttataacgatgcggtgcgcaacaccacggcgatttggaacgaaaccccggtggatctgggcaaccgccaggcgtggtttgaagcgcgcgcgcagcagggctatccgattctggtggcggtggatcatagcggcgtgctgggctatgcgagctttggcgattggcgcccgtttgaaggctttcgcaacaccgtggaacatagcgtgtatattcgcggcgatcagcgcggcaaaggcctgggcccgcagctgatgaccgcgctgattgcgcgcgcgcgcggctgcggcaaacatgtgatggtggcggccattgaaagcggcaacgcggcgagcgtgcgcctgcatgaacgcctgggctttgtggtgaccggccagatgccgcaggtgggcgtgaaatttggccgctggctggatctgacctttatgcagctggtgctggatccgggcgcggaaccggcgtga

SEQ ID NO: 8 - DNA, 492 bp, Bacillus subtilis
atgaccctgcgcctggcggaacatcgcgatctggaagcggtggtggcgatttataacagcaccattgcgagccgcatggtgaccgcggataccgaaccggtgaccccggaagatcgcatggaatggtttagcggccataccgaaagccgcccgctgtatgtggcggaagatgaaaacggcaacgtggcggcgtggattagctttgaaaccttttatggccgcccggcgtataacaaaaccgcggaagtgagcatttatattgatgaagcgtgccgcggcaaaggcgtgggcagctatctgctgcaggaagcgctgcgcattgcgccgaacctgggcattcgcagcctgatggcgtttatttttggccataacaaaccgagcctgaaactgtttgaaaaacatggctttgcggaatggggcctgtttccgggcattgcggaaatggatggcaaacgctatgatctgaaaattctgggccgcgaactgagctga

SEQ ID NO: 9 - DNA, 516 bp, Enterobacter sp. 638
atgatcatccgccatgccagtaaagaagattgcgccgctatcggcgagatttataaccacgccgttgtgcacactgccgctatctggaatgacaccaccgttgataccgagaaccgcattgcgtggtttgaagctcgcacgttgatggggtatccggtgctggtcagtgaagaaaatggcgtggtcacgggctatgcgtcatttggcgactggcgtgcatttgacggatttcgccatacggtcgaacattcggtctacgttcaccccgaccatcagggcaaaggaattggccgtgagctgatgaaagcgctgattggtgaagcgcgaaacatcggcaaacacgttatggtggcgggaattgaggcacaaaatcacggctcaattcacctgcataagacgctcggatttgtgattaccgggcaaatgccgcaggtcgggaccaaatttggccgctggctggatctcacctttatgcagctccagcttgacgagcgcatcgacccggacgctatctga

SEQ ID NO: 10 - DNA, 528 bp, Pseudovibrio sp. FO-BEG1
atgaaactgcgtcaggcaaccaaatctgatcttccgacacttctggaaattcacaatgatgccgttaagacactagctgcgatttggacggatactttagagacgctggaagatcgagtgagttggttcgaaaagcggatcgcaggcgggtttccgatcattgtagctgaagatgagaacggcgatgtacttggctacggcagttacggatcttttcgtgaaaaatctggttacgataagacggtggagcattctgtctacgtaaccccgcaatcacgcggtaacggtgctggctccgttttgctggaaaagctgatcgaactggcaaaacaggatgatcgccatgtccttattggcgcaatcgacagtgaaaacaaaggctcaatccgcctccatgaacgctatggcttcaggatcaccggagaactcccacaagtcggcttcaaattcggccgctggctggatctcaccctgatgacgcttatcttaaacgatgatgaagcaccaacagcactcgcgcatgaataa

SEQ ID NO: 11 - DNA, 465 bp, Yarrowia lipolytica PO1f
atgaagatatctccagaaccctacaccgccgatttgtacaaattggtgcgcaaaaacatgaagggaatgtacgagggttcggggatggggtggaatagggttgacaagattgacgagatggaggacgaggagctggcgtatcacgtggctcgcgaaaatggagagatgctaggattcgtctcgttcatgcatacggttgaagacgacgtggaggtggtatatctgtatgagcttcaggtggccaagggtcgccagggtcacggtgtgggtaaggagctcatgagggttgtgatagacgaggctagggcttgtggtcgtccgatcatgttgactgtttttctcatgaatgagcgggccattggtttctacaggcggtatggttttgagcgggtggggcggggtcctcaggagggcaagcgggtgaggggatggatgcagatgaggcgagacacgaggagtgactag

SEQ ID NO: 12 - DNA, 540 bp, Corynebacterium glutamicum ATCC 13032
atggttgaaagagacttcactatccgaccaatccgcgagggtgatttccctcaggtgagggacatctacgaattgggcctggagacgggacatgcgacttatgagacttctggtcccacgtgggaccagttctcccaatctaaaatcatggataccgtcatggtggcggtagaaaacaacgacccggacttcatcctcggatgggtgtctgctgctccaatttcaagccgacaggttttccatggagtggtggaagattccatctatatccacccccagggccaaggccgaggaatcggcggcgctttgctcgacgcccttatcacctactgcgaaagcaacggcatctggtcgatccactcctggatcttcccggaaaacctcggttctgcgaaactgcatgaatcgaagggcttcgtgaaggtgggcaccatgcaccaaatggcaaggatgccctacggcgagatggaaggacaatggcgcgattgtgatctgtgggagtgcctcttatccgttccagagcaagctcaaagttcctaa

SEQ ID NO: 13 - DNA, 27 bp, Artificial Sequence
  primer 1
atccatatgaagatatctccagaaccc

SEQ ID NO: 14 - DNA, 27 bp, Artificial Sequence
  primer 2
tactctagactagtcactcctcgtgtc

SEQ ID NO: 15 - DNA, 26 bp, Artificial Sequence
  primer 3
atccatatggttgaaagagacttcac

SEQ ID NO: 16 - DNA, 27 bp, Artificial Sequence
  primer 4
tactctagattaggaactttgagcttg

SEQ ID NO: 17 - DNA, 18 bp, Artificial Sequence
  primer 5
atcatgagccatgaaatt

SEQ ID NO: 18 - DNA, 24 bp, Artificial Sequence
  primer 6
gcactgcagtcacgccggttccgc

SEQ ID NO: 19 - DNA, 18 bp, Artificial Sequence
  primer 7
atcatgaccctgcgcctg

SEQ ID NO: 20 - DNA, 24 bp, Artificial Sequence
  primer 8
gcactgcagtcagctcagttcgcg

SEQ ID NO: 21 - DNA, 18 bp, Artificial Sequence
  primer 9
atcatgatcatccgccat

SEQ ID NO: 22 - DNA, 24 bp, Artificial Sequence
  primer 10
gcactgcagtcagatagcgtccgg

SEQ ID NO: 23 - DNA, 18 bp, Artificial Sequence
  primer 11
atcatgaaactgcgtcag

SEQ ID NO: 24 - DNA, 24 bp, Artificial Sequence
  primer 12
gcactgcagttattcatgcgcgag

SEQ ID NO: 25 - DNA, 18 bp, Artificial Sequence
  primer 13
atcatgaagatatctcca

SEQ ID NO: 26 - DNA, 24 bp, Artificial Sequence
  primer 14
gcactgcagctagtcactcctcgt

SEQ ID NO: 27 - DNA, 18 bp, Artificial Sequence
  primer 15
atcatggttgaaagagac

SEQ ID NO: 28 - DNA, 24 bp, Artificial Sequence
  primer 16
gcactgcagttaggaactttgagc

SEQ ID NO: 29 - DNA, 24 bp, Artificial Sequence
  primer 17
tgcactagtatgagccatgaaatt

SEQ ID NO: 30 - DNA, 24 bp, Artificial Sequence
  primer 18
tgcctcgagtcacgccggttccgc

SEQ ID NO: 31 - DNA, 24 bp, Artificial Sequence
  primer 19
tgcactagtatgaccctgcgcctg

SEQ ID NO: 32 - DNA, 24 bp, Artificial Sequence
  primer 20
tgcctcgagtcagctcagttcgcg

SEQ ID NO: 33 - DNA, 24 bp, Artificial Sequence
  primer 21
tgcactagtatgatcatccgccat

SEQ ID NO: 34 - DNA, 24 bp, Artificial Sequence
  primer 22
gcactgcagtcagatagcgtccgg

SEQ ID NO: 35 - DNA, 24 bp, Artificial Sequence
  primer 23
tgcactagtatgaaactgcgtcag

SEQ ID NO: 36 - DNA, 24 bp, Artificial Sequence
  primer 24
tgcctcgagttattcatgcgcgag

SEQ ID NO: 37 - DNA, 24 bp, Artificial Sequence
  primer 25
tgcactagtatgaagatatctcca

SEQ ID NO: 38 - DNA, 24 bp, Artificial Sequence
  primer 26
tgcctcgagctagtcactcctcgt

SEQ ID NO: 39 - DNA, 24 bp, Artificial Sequence
  primer 27
tgcactagtatggttgaaagagac

SEQ ID NO: 40 - DNA, 24 bp, Artificial Sequence
  primer 28
tgcctcgagttaggaactttgagc

SEQ ID NO: 41 - DNA, 24 bp, Artificial Sequence
  primer 29
tgcggtaccatgagccatgaaatt

SEQ ID NO: 42 - DNA, 24 bp, Artificial Sequence
  primer 30
ctaggtacctcacgccggttccgc

SEQ ID NO: 43 - DNA, 24 bp, Artificial Sequence
  primer 31
tgcggtaccatgaccctgcgcctg

SEQ ID NO: 44 - DNA, 24 bp, Artificial Sequence
  primer 32
ctaggtacctcagctcagttcgcg

SEQ ID NO: 45 - DNA, 24 bp, Artificial Sequence
  primer 33
tgcggtaccatgatcatccgccat

SEQ ID NO: 46 - DNA, 24 bp, Artificial Sequence
  primer 34
ctaggtacctcagatagcgtccgg

SEQ ID NO: 47 - DNA, 24 bp, Artificial Sequence
  primer 35
tgcggtaccatgaaactgcgtcag

SEQ ID NO: 48 - DNA, 24 bp, Artificial Sequence
  primer 36
ctaggtaccttattcatgcgcgag

SEQ ID NO: 49 - DNA, 24 bp, Artificial Sequence
  primer 37
tgcggtaccatgaagatatctcca

SEQ ID NO: 50 - DNA, 24 bp, Artificial Sequence
  primer 38
ctaggtaccctagtcactcctcgt

SEQ ID NO: 51 - DNA, 24 bp, Artificial Sequence
  primer 39
tgcggtaccatggttgaaagagac

SEQ ID NO: 52 - DNA, 24 bp, Artificial Sequence
  primer 40
ctaggtaccttaggaactttgagc